European Patent Application EP 4 389 886 A1, published June 26, 2024. Title: LACTASE ENZYMES AND METHOD OF PRODUCING A MILK-BASED PRODUCT. Applicant: Novozymes A/S. The sequence listing filed with the application follows.

SEQUENCE LISTING (15 sequences)

SEQ ID NO: 1 - protein, 1298 aa, Bifidobacterium samirii
DDILSRADSTTQMSSDPEVVYANAVTGTAERSMNFDANWRFLLSDSVSAQDPGFDDSQWRQISLPHDYSIEQDYSTSGEAESAYLPGGTGWYRKQFTLSRDLAGKRVSIGFDGVYMNATVWINGHKLGTHPYGYSPFSFDLTDHAVFGGENTIVVKVENKTPSSRWYSGSGIYRSVTLNVTDAVHVDTGGVRVTTPDLAAQHGGDVTVNLGADIANDSGAPVEVTLRQSVFAKGEGTERAIGTSVGEPTTIAAGASAHIDSTLTASSPKLWSTQNPNLYTVRTEVMSGDTVLDTYDTDYGFRWTSFDADGGFSLNGTPTKIKGVSMHHDQGALGAVANRRAIERQVEILKGMGVNSIRTTHNTAARTLIDVCNEQGVLVVEEAFDTWIKAKNGNSEDYGKWFSVEVGDGNAIEGGDASGTWALFDLTAMIRRDANDPSVIMWSLGNEMMEGISGSVSEYPDVARRLIAWTNEADPTRPATLGDNKIKAGWSESTAMADALTDSDGVVGTNYSSGGNYDSVHAAHPDWRLYGSETASAINSRGIYDRTTGGSQTADKQLTSYDASAVGWGATASSAWYDVITRDFVAGEYVWTGFDYLGEPTPWNGTGSGAQGAWPSPKSSYFGIVDTAGLPKDSYYFYQSQWNDDVHTLHVLPAWNENVVAKDSQGKVPVVVYSDAAAVELFFTPKGGERTSLGRRQFTTKTTAAGYRYQVYEGEGKSSSADKNLYLTWNVPWAEGTITAVAYDESGAVIADTEGRSSVTTTGEASALTAEADRTTIEADGTDLSYVTVDVTDADGNTVPDAADRVTFDVKGAGRLVGVDNGSSPDHDSYQANNRRAFSGRLVAIIQSTDKAGDITVTATADGLKSSTTTITTTAVPGASTERAVDGLYYARNYYVKTGNSPRLPDTIEVRYTDGTSERQAVTWNEVGDDQTAVPGTFTVTGTVGEQTATVRVTMIDDGGALLNYSATTPVGIAPALPESRPLVLADGTVTNAGFAVSWTTPDDSAYAEAGTVTVPGTATVFDRTVDVSATIRVQQESVAIGDSVSGSALNLTQSVPADLQTDTLDAIKDGSATADPNTGGGANPSVWTNYNWAQSGRDGSDKSELTFEYATQQKFGRFVMHFYTDSYSARLPKNVDIQVSDDGANWTTLSTTATKGETRDNVTPYTYDFAPVTATFVRFAITNSDEALSGRRPCTGISEIELKLAVTDFTTNTDAGLSSLTVNGTDVPASALAAGSWNTPAIRADVEAVGAGNASVTVLPAHEGVIRVITESEDHATRGVFAVNLGREQSDAADSDA

SEQ ID NO: 2 - protein, 1288 aa, Streptococcus entericus DSM 14446
TESPEEWHKVNHYNDTDKVVNFDKDWKFNLGDSAAASSKSFDDSSWKKLDLPHDFSLIQDYTPSGEAESGYKPGGIGWYRKSFTIGEEAAKGRVNLQFDGAYMETEVFINGTSLGTHTYGYSPFSFDLTEHLKKDEENVLAVKVTNPIPSSRWYSGSGIYRSVHLEFAPSVHLAEYGVVVTTPDLKDTHNLDSGSRINISTTVVNQGEDAAQVTVRSTLFERDSNGGRGRQVAVSTDVPAKSVTAGSSSAIDTSLTIVKPKLWSVDNPHLYVLRTEVLKDGQVIQSREQETGFRYTAFDKDTGFKLNGQNLKLQGVSMHHDQGGLGARAYYDAIERQFTILKDMGVNAVRVTHNPASRAMKDIANRKGMLLIDEAFDTWEHAKNGNTNDYARYFNRVIGDSVRDLNGARADQTWAEYHIKQMVKSGINDPSIIMWSTGNEVMEGFSANTSNYPQVIARLSDWVAEIDPTRPATFGDNMLKNRHQNAIGMANVLTEKKGIVGYNYANGAQYDQGHRDHPDWIIYGSETASAVNSRGVYNVKGNTQRQDRQLTSYDQSKVNWGHVASEAWYDVLTRDFVAGEFVWTGFDYLGEPTPWNKTNPGAQGTWGSPKSSYFGIVDTAGLPKDSYYFYRSQWQKGDTTLHVLPAWEESVVAKDNQNRVEVVVYSNAAKVKLVHISPEGVERVIGTKAFSKETTSAGHTYQVYKGSDKQQVEHKNLYLTWHVPYEAGTIKAIALDEQDRVIEQTVGTSQVSTFGAAHKLQATVTHKKDTVDDHNLAYVTIDVQDAKGNLVVNASNRIKVTVTGEAELVAMDNGNPVDHQSYQDDNRQAFGGKVVAILKMTGKAGQVQVTATADGLASSTQTFEVAAKRQSQADKVDSYKLTKTIYIKKGAELKLPEKTTVRYEDGREVEKDLHFDRSAIAPKLAAGETFTATGRINDLGTRAELVVAVIDQVAAIKNISTATEVGARPKLPETAQAYLADGSLLSATFPVSWQMPEEAQFAQTGTVMINGTADVLGQKLPITASVRVGEKTLTIDQNVAPSARTLTQNIVGSDTLTAINDGNLNVSANNQGGPNPTIWSNWQAAQNGQKTATLSFTYDTAQTIAEVVAYYHRDRLSLRTPKSATFAWNRGSGAEDETIAIASQTAEAVAGTSLTKVTYRLAQPVSAVEFKMTVENSDEAMPSAQKSSVGIAEVQLMTALESFNQHSEAGLTDIRVGDRRYTGNQISTSMRVPATGAVTATNNNRNVGITILPEQDGVVKIFTESEDKTRSAVYSIQLVPENPRTPDD

SEQ ID NO: 3 - protein, 1309 aa, Varibaculum sp.
AGNTDYSHLNTSAQMVSSAQSVPLTTIDGKSRFQSLNNGWKFNLGDISGAQATAYNDAKWRTVDIPHDYSIEQPFSKSMEGESGYLPGGVGWYRKSLNLPSELQHKRIKLSFDGIYMDATIYVNGTELANHPYGYTPFSIDITDNVKFGENNVIAVKVNHQTPSSRWYSGSGIYRDVDLVITDPIHIASSGVKITPKNIDTYTEAGSLDLDLSTKIINAAASPKTITLRHTISPKTGGNSIGTVTSTPITVEAGKSLTNSTALSAQSPQLWTIEKPVQYLVKTEVFEGSRLLDTLETNTGFRQLTFDPNTGFALNGKKMKLKGVSMHHDQGALGAKAYRDAIARQIDILKKMGANTIRITHNPASRDLIDLANQKGMLLIEEIFDGLHCTKNGNQMDYARFFNQLVPKDSKLENVTAGSTWARFDLETTMRRDINAPSIIMWSLGNEIQEGTTCGIDSFLSPQTNLIKWAAEIDNTRPLTRGDNAIKHNNSAINVMKSLVSTAKTSGTTGAVGANYANGGQYDSIHRQIPGAMLYGAETASSVNSRGVYSRTTDNRQTADKQLTSYDNSKVNWGATAAQAWLDVIKRDFVAGTAVWTGFDYLGEPTFWNGTSPGPQGQWPSPKNSYFGIIDTAGFPKDSYYLYQSQWNDKVTTLHVLPAWNRSILQNQGNGNQKVVVYSDASAVELFFTGTDGKKKSLGKKTFAKKTTPAGYKYQLYEGSDKSSIESENLYLSWNVQYADGTLSAVAYDESGNVITNTQGRDTVSTAGKAAKLDVSLNRTELSANNQDLAYVEVTVIDDNGTPVPDANLKVDFNASGACEMMGTDAGKQDDHTSYLSSSRNTYNGKVLGIVKSKKIAGQCTINVSGTNLPKVTKTITVTPAPNASQDRAIDAYSYPRNYYVQVGTQPRFPDKIDAIFTDGSQDAVEVTWNQVPKEQYSKAGFFTVLGKTKHGHQVSANVTMLNRVGAVLNYSATTPVGIVPTIPATRPAVLPDGTILDVQFDVTWQKPNEKVYSKAGTVTIEGKAKFLDKELPVTATIRVQEAVVKIGDSVSGAATLSQDIPADKQSDTLDAIKDGNTAVGSNTQGGANPTAWTNYTNSQAGDNSAAIEFKYATQQTFGEFNVYFFKDSYSARYPDGGTTKFYVKEAAGDQWKPVETTESIATSEHPENVKKYSYALKKPVNATYVKLEVINKSEQLSGHNPCTGITEVELKTASNTTSTFSTAKLASLQVNGENLSKSVLKSFEYATPAEKITQIKALAKDNAAITVLPEYEGVARVIIESEDHKTINIFKIYLGKEQPEPADDASRD

SEQ ID NO: 4 - protein, 1307 aa, Urmitella timonensis
AGNTDYSHLNTSAQMVSSAQSVPLTTIDGKARFQSLNNGWKFNLGDISGAQATAYNDAKWRTVDIPHDYSIEQPFSKSMEGESGYLPGGVGWYRKSLNLPSELKNKRIKLSFDGIYMDATIYVNGTELANHPYGYTPFSIDITDNVKFGGNNVIAVKVNHQTPSSRWYSGSGIYRDVDLVITDPIHIASSGVKITPKNIDTYTEAGVLNLDVSTKLINAATSPKTITLRHTISPKNGGNSIGTVTSTPITVEAGQSLTDSTALSAQSPQLWTIEKPVQYLVKTEVFEGSKLLDTLETNTGFRQLTFDPNTGFALNGKKMKLKGVSMHHDQGALGAKAYRDAIARQIDILKKMGANTIRITHNPASRDLIDLANQKGMLLIEEIFDGLHCAKNGNQMDYARFFNQLVPKDSKLENVTAGSTWARFDLETTMRRDINAPSIIMWSLGNEIQEGTTCGIDSFLSPQTNLIKWAAEIDNTRPLTRGDNAIKHNNSAINVMKSLVSTAKTSGTTGAVGANYANGGQYDSIHRQIPGAMLYGAETASSVNSRGVYSRTTDNRQTADKQLTSYDNSKVNWGATAAQAWLDVIKRDFVAGTAVWTGFDYLGEPTFWNGTSPGPQGQWPSPKNSYFGIIDTAGFPKDSYYLYQSQWNDKVTTLHVLPAWNRSVLQNQGNGNQKVVVYSDASAVELFFTGTDGKKKSLGKKTLAKKTTPAGYKYQLYEGSDKSSIESENLYLSWNVQYADGTLSAVAYDESGNVITNTQGRDTVSTAGKAAKLDVSLNRTELSANNQDLAYVEVTVTDDNGTPVPDAALKVDFNASGACEMVGTDAGKQDDLTSYLSSSRNTYNGKVLGIVKSKKIAGQCTITVSGTNLPKVTKTVTVTPAPNASQDRAIDAYSYPRNYYVQVGTQPRLPDKIDAIFTDGSQDAVEVTWNQVPKEQYSKAGFFTVLGKTKHGHQVSANVTMLNRVGAVLNYSATTPVGIVPTIPATRPAVLPDGTILDVQFDVAWQKPNEKVYSKAGTVTIEGKAKFLDKELPVTATIRVQEAVVKIGDSVSGAATLSQDIPADKQSDTLDAIKDGNTAVGSNTQGGANPTAWTNYTNSQAGDNSAAIEFKYATQQTFGEFNVYFFRDSYSARYPDGGTTKFYVKEAAGDQWKPVETTESIATSEHPENVKKYSYALKKPVNATYVKLEVTNKSEQLSGRNPCTGITEVELKTASNTTSTFSTAKLASLQVNGENLSKSVLKSFEYATPAEKITQIKALAKDNAAITVLPEYEGVARVIIESEDHKTINTFKIYLGKEQPEPADDAS

SEQ ID NO: 5 - protein, 1304 aa, Bifidobacterium bifidum
VEDATRSDSTTQMSSTPEVVYSSAVDSKQNRTSDFDANWKFMLSDSVQAQDPAFDDSAWQQVDLPHDYSITQKYSQSNEAESAYLPGGTGWYRKSFTIDRDLAGKRIAINFDGVYMNATVWFNGVKLGTHPYGYSPFSFDLTGNAKFGGENTIVVKVENRLPSSRWYSGSGIYRDVTLTVTDGVHVGNNGVAIKTPSLATQNGGNVTMNLTTKVANDTKAAANITLKQTVFPKGGKTDAAIGTVTTASKSIAAGASADVTSTITAASPKLWSIKNPNLYTVRTEVLNGGKVLDTYDTEYGFRWTGFDATSGFSLNGEKVKLKGVSMHHDQGSLGAVANRRAIERQVEILQKMGVNSIRTTHNPAAKALIDVCNEKGVLVVEEVFDMWNRSKNGNTEDYGKWFGQAIAGDNAVLGGDKDETWAKFDLTSTINRDRNAPSVIMWSLGNEMMEGISGSVSGFPATSAKLVAWTKAADSTRPMTYGDNKIKANWNESNTMGDNLTANGGVVGTNYSDGANYDKIRTTHPSWAIYGSETASAINSRGIYNRTTGGAQSSDKQLTSYDNSAVGWGAVASSAWYDVVQRDFVAGTYVWTGFDYLGEPTPWNGTGSGAVGSWPSPKNSYFGIVDTAGFPKDTYYFYQSQWNDDVHTLHILPAWNENVVAKGSGNNVPVVVYTDAAKVKLYFTPKGSTEKRLIGEKSFTKKTTAAGYTYQVYEGADKDSTAHKNMYLTWNVPWAEGTISAEAYDENNRLIPEGSTEGNASVTTTGKAAKLKADADRKTITADGKDLSYIEVDVTDANGHIVPDAANRVTFDVKGAGKLVGVDNGSSPDHDSYQADNRKAFSGKVLAIVQSTKEAGEITVTAKADGLQSSTVKIATTAVPGTSTEKTVRSFYYSRNYYVKTGNKPILPSDVEVRYSDGTSDRQNVTWDAVSDDQIAKAGSFSVAGTVAGQKISVRVTMIDEIGALLNYSASTPVGTPAVLPGSRPAVLPDGTVTSANFAVDWTKPADTVYNTAGTVKVPGTATVFGKEFKVTATIRVQRSQVTIGSSVSGNALRLTQNIPADKQSDTLDAIKDGSTTVDANTGGGANPSAWTNWAYSKAGHNTAEITFEYATEQQLGQIVMYFFRDSNAVRFPDAGKTKIQISADGKNWTDLAATETIAAQESSERVKPYTYDFAPVGATFVKVTVTNADTTTPSGVVCAGLTEIELKTATSKFVTNTSAALSSLTVNGTKVSDSVLAAGSYNTPAIIADVKAEGEGNASVTVLPAHDNVIRVITESEDHVTRKTFTINLGTEQEFPADSDERD

SEQ ID NO: 6 - protein, 1313 aa, Bacillus sp. S3
AEKTNASTENSVTYEGERRINFNGNWRFQRETTGSIAGAQNPGFDDSSWRQLNLPHDWSIELDFNKNSLATHEGGYLDGGIGWYRKTFTVPESMKGKRISIDFDGVYMNSTTYLNGQLLGTYPFGYNAFSYDITDKLYRDGRENVLVVKVNNTQPSSRWYSGSGIYRNVYLTVTNPVHVARYGTFVTTPNLETAYAAGKADVNIKTKVSNDSGEAVQVKVKSTIYDDAGKAVATVESEEKTAAAGAETQFENNTIIEQPKLWDIDNPYRYKLVTEVIARGQSVDTYETRFGARYFNFDENEGFSLNGKYMKLHGVSMHHDLGALGAATNARAVERQMQIMKDMGVNAIRVTHNPASPELLEAANKLGLFIVEEAFDSWAQSKKTYDYGRFFTTWAEHDIKEMVDRGKNEPAIIMWSIGNEIYDTTNAAGVETARNLVRWVKEIDTTRPTTIGEDKTRGDKVNVTPINSYIKEIFNIVDIVGLNYSENNYAGYHQQNPNWKLYGSETSSATRSRGVYTHPYQYNQSTKYADLQQSSYDNDYVGWGRTAEDAWKYDRDLKHIAGQFIWTGFDYIGEPTPYYNAYPAKSSYFGAVDTAGFPKDIFYYYQSQWKKEPMVHLLPHWNWTEGETVRVLAYTNAYKVELFLNGESLGVRSYENKKTSWGAPYKETKDGKTYLEWAVPFKAGTLEAVAKDESGKEIARDQVVTAGEPAAVKLTADHKVITADGTDLSFITAEIVDSKGIVVPNADHLIKFNVSGQGELAGVDNGNASSVERYKDNKRKAFSGKALAIIQSNKLAGEITVNASVAGLSGDTTSLFTVAPADRDKKTVVGMDTVHVTIDVDQAPKLPTELKVYYSDATVDAKKVTWDLVDPKQYSSVGIFTVEGKVEGTSLKAKAVVTVKGIVAVKPVSTATKVGVRPVLPENVALLYSDETTKDVNVSWEEISADQLAKEGRFVVEGSVEGTDLKAKAFVRVTNESKPVNIMLPAQGSTYPQLEATFTNPADNLQHLNDGIKSYTNSPVNRWTNWTRTPRDAGDSITVNFGKQHVINNLDLFVFTDSGTVVPDTAAVQYWDGTAWKDVENLTQPSPYVVEKNEIRFDAVTTDKLKFHLIPSVKGKYLALTEAEIFADQMVMSSTASLSSIIVNGKPLAGFDAAKKTYDLVLPYGSDLPKIEAEAADNAAVTILPAFTYPGTAKLFVTSEDGKVTSEYSIQVSMEEPKLVAAKLSVDQTKVVEDDIIDLKVEGTLESGEVIDLTDSEPTYEFDNQNIKIEGNKLYALETGEVKVKAVVKYKDVTVTTPEMTISIAKNPAPKYI

SEQ ID NO: 7 - protein, 1299 aa, Bifidobacterium aerophilum
DDTATRADSTTQMSSTPEMVYANRVEADQARTTDFDANWKFKMSDAIAAQDPDFDDSAWQRISLPHDYSITQDYTQSGEAESAYLPGGTGWYRKTFTLDRGLAGKQVSVNFDGVYMNATVWLNGVKLGEHPYGYSPFSFDLTKAARFGAENTIVVKVDHKTPSSRYYSGSGIYRDVTLTVTDGVHVAGNGVAVATPELAEQNGGDVTMNLTATVSNDTEAAADVTLKQTVFPKGGETSAAIGTVITEATNVAAGESADVASTITAAQPKLWSVENPNLYTVRTEVQVAGRTVDTYDTTYGFRWTGFDADTGFSLNGVKVKLKGVSMHHDQGSLGAVANHSAIARQVRILKDMGVNSIRTTHNTAAKALIDICNEEGILVIEEIFDGWNRAKNGNTEDYAKYFDKTIASDNRILGGDKDESWAKFDLTATINRDRNDPSIIMWSTGNEMMEGISGGVSDFPDISAKLTRWTNAADATRPATYGDNKIKANWTESNTMGDSLTAAGGVVGANYEDGRLYDSTHQAHPTWKLYGSETASSINSRGIYNVTTGATGDQQLTSYDNYAVGWGATASSAWYDVIRRDFVAGEYVWTGFDYLGEPTPWNGTDSGFKGTWPSPKNSYFGIVDTAGLPKDSYYFYRSQWNTKSHTLHILPAWNGDVVAKDSSGNVPVVVYTDAATVKLYFTPKGSSDKRLIGEKSFTTHTTDAGYTYQTYDGADKNATADKNMYLTWNVKWAEGTITAEAFDKDGRRITDTEGRSRVTTTGVASQLKVEADATKLTADGKSLSYITVDVTDADGNVVPNADDRVTFKVEGAGKLVGVDNGKTTDHQSYQDDNRKAFSGKLVAIVQSTKTAGGITVTATAEGLKPATTTITTTAVPGASTARTIDGFYYARNYYVKTGNKPMLPSDVEVRYSDGTKDRQNVTWNVVTDEASKTGTFTVTGTVADQTISVRVTMIDEGGALLNYSATTQVGMPAVLPESRPLVLSDGTVTSANFAVTWTKPADGEYDEAGTVVVPGIATVFGKEIGVTATIRVQTANVTIGDSVSGNAMNLTQDIPEGSQSDTLDAIKNGSTTVDDNLSGGANPSAWTNWAWSKAGHNTAQITFEYATQQTLGQIVMYFFRDSSSVTFPDAGTTKIEISDNGTDWTRLNVEETIAPAESSNRVKPYTYDFAPTGATFIRFTVTNSETRASSGVTSTGLTEIELKVATTTFTTNTAAGLASLKVNGTAVSESALASGSYNTPAIVADVEAVGKDNASVTVLPAHNDVIRVITESEDHATRETFAINLGKEQEDTADSDARD

SEQ ID NO: 8 - protein, 1304 aa, Bifidobacterium mongoliense
VEDATRSDSTTQMSSTPEVVYSSAVDSKQDRTSDFDANWKFMLSDSVQAQDPTFDDSAWQQVDLPHDYSITQKYSQSNEAESAYLPGGTGWYRKSFTIDRDLAGKRIAINFDGVYMNATVWFNGVKLGTHPYGYSPFSFDLTGNAKFGEENTIVVKVENRLPSSRWYSGSGIYRDVTLTVTDGVHVGNNGVAIKTPSLATQNGGDVTMNLTTKVANDTKAAANITLKQTVFPKGGKTDAAIGTVTTASKSIAAGASADVTSTITAASPKLWSIKNPNLYTVRTEVLNGDTVLDTYDTEYGFRWTGFDATSGFSLNGEKVKLKGVSMHHDQGSLGAVANRRAIERQVEILQKMGVNSIRTTHNPAAKALIDVCNEKGVLVVEEVFDMWNRSKNGNTEDYGKWFGQTIAGDNAVLGGDKDETWAKFDLTSTINRDRNAPSVIMWSLGNEMMEGISGSVSDFPATSAKLVAWTKAADSTRPMTHGDNKIKANWNESNTMGDNLTANGGVVGTNYSDGANYDKIRKNHPSWAIYGSETASAINSRGIYNRTTGGAQSSDKQLTSYDNSAVGWGAVASSAWYDVVQRDFVAGTYVWTGFDYLGEPTPWNGTGSGAVGSWPSPKNSYFGIVDTAGFPKDTYYFYQSQWNDDVHTLHILPAWNENVVAKDSGNNVPVVVYTDAAKVKLYFTPKGSTEKRLIGEKSFTKKTTAAGYTYQVYEGANKNSTVHKNMYLTWNVPWAEGTISAEAYDENNKLIPEGSTEGNASVTTTGEAAKLKADADRKTITADGKDLSYIEVDVTDANGHIVPDAANRVTFDVKGAGKLVGVDNGSSPDHDSYQADNRKAFSGKVLAIVQSTKEAGEITVTAKADGLQSSTVKIATTAVPGTSTEKTVRSFYYSRNYYVKTGNKPILPSDVEVRYSDGTSDRQNVTWDAVSDDQIAKAGSFSVAGTVAGQKISVRVTMIDEIGALLNYSATTPVGTPAVLPGSRPAVLPDGTVTSANFAVDWTKPADTVYNTAGTVKVPGTATVFGKEFKVTATIRVQRSQVTIGSSVSGNALRLTQNIPADKQSDTLNAIKDGSTTVDANTGGGANPSAWTNWAYSKAGHNTAEITFEYATEQQLGQIVMYFFRDSNAVRFPDAGKTKIQISADGKNWTDLAATETIAAQESSDRVKPYTYDFAPVGATFVKVTVTNADTTTPSGVVCAGLTEIELKTATSKFVTNTSAALSSLTVNDTKVSDSVLAAGSYNTPAIIADVKAEGEGNASVTVLPAHDNVIRVITESEDHVTRKTFTINLGTEQEFPADSDERD

SEQ ID NO: 9 - protein, 1291 aa, Clostridium nexile CAG:348
SGQVQVRTDSNTQMSSDKEVVYVNTYDTSKRVHDFDANWKFYLGDADGAEAVNFDDSAWRTVSVPHDYSIEQEYTQSGEAESGYLPGGTGWYRKHFTLTEDMKDKEIRLDFGGVYMNATVWVNGTQLGTHPYGYTPFSFDITDYVKAGEENVITVKVDHQTPSSRWYSGSGIYRSVDLTVMDKVHVDLNGTKIATPNLAKEKDGDVNMDIVTTVANEEKEAKEIILVHTLREKGKKDAVATVTTERQSVEAGKTAGIKANLKVNQPKLWGLGEKNAHLYTVTTEVKVNDKVVDTYDTDYGFRYTELDTKTGFSLNGEKVKLQGVCMHHDQGALGAEAQKRAIERQVEILQEMGCNSIRVTHNPAAEELIEVCNEKGILVINELFDGWHKAKNGNVNDYAKWFNQTIGDENKILDGKSDMTWAEFDLKSTLNQGKNDPSIIMWSLGNEISEGASEGGYYEISKNLIKWAQEIDTSKPLTIGSNRVKGAIGQADNEHIKIANDLTKIGGMSGTNYSGGSNYDALHSTYPEWFLYGSETASAVNSRGVYTTKANAALDQDKQLTSYDKSKVNWGALASEAWYDVITRDFVAGEYVWTGFDYIGEPTPANKINAGAATSWPSPKNSYFGIVDTAGLPKDSYYFYQSQWNDEVNTLHVLPTWNEDSLMKDENGNVEVVVYSDAAKVKLFLNDKEIAEQTFEEHTTGAGYKYQTVKGKTGHESMYMTFSVPYEKGTLKAVAYDKDGNEIKNTQGRSSVTTTDKATKLDATVDRNSIKADGKDLSYITVDVTDANGNIVPDADNNVRFTVEGAGTLVGVDNGKQADHQSYQDDNRDAYNGSLVAIVQSTKDAGKITVKAEADGLTLDTVEITTTEVEDGTVDKTQVDSFYMSKHYYVKAGSKVQLPETIKTRFKDGTEKDLPVKWDEIKETTGSFVVNGLVDGKYKVSVTVNVIDQLGGLMNYSATTPKGTEPNLPTTRPAIAQDGTVLNVSFPVTWGKVDKTKYDEPGIVTVNGTSNVLGTAMEVTASIRVQEETYEIVGSVDNPSQLTQDIEKDKQSDTLDAVWDGKTAIADNTSGGPNPTAWSNYKNSQAGDNTAEITFQYATQQVIGEVTVHFFKDSASARYPKAGTTKLYVKANDGDDWQEVVAEETIGEENGRVKAYTYKFNPVGATLFKVAVTNSDEVLTTGHKPCTGITEIEIKKAVGSYKTNTTAKLASLEVNGKALTAEELAENAYYTLDKTATVTAAGADNAAVTVLPVHNKQIRILIESEDHRTKNTFVIYLEQEKPMSPDDDSKD

SEQ ID NO: 10 - protein, 1130 aa, Neobacillus bataviensis
AEKTNATTENSLHFEGERRMNFNGNWRFQRETNGSIAGVQNPGFDDSSWRQLNLPHDWSIELDFNKNSLATHEGGYLDGGIGWYRKTFSVPAAMKGKRISIDFDGVYMNSTTYLNGQLLGTYPFGYNAFSYDITDKLYTDGRENVLVVKVNNTQPSSRWYSGSGIYRNVYLTVTNPVHVARYGTFVTTPNLETASAAGKADVNIKTKISNDSGEAAQVKVKSTIYDEAGKAVSTVESEGKTAAAGAEAHFENNTIIEQPKLWSIDNPYRYKLVTEVIVGGQTVDTYETRFGARYFKFDENEGFSLNGKYMKLHGVSMHHDLGALGAATNARAVERQMQIMKDMGVNAIRVTHNPASPELLEAANKLGLFIVEEAFDSWAQSKKTYDYGRFFTTWAEHDIKEMVDRGKNEPAIIMWSIGNEIYDTTNAAGVETARNLVRWVKEIDTTRPTTIGEDKTRGDKVNVTPINSYIKEIFNIVDIVGLNYSENNYAGYHQQNPNWKLYGSETSSATRSRGVYTHPYQYNQSTKYTDLQQSSYDNDYVGWGRTAEDAWKYDRDLKHIAGQFIWTGFDYIGEPTPYYNAYPAKSSYFGAVDTAGFPKDIFYYYQSQWKSEPMVHLLPHWNWTEGESVRVLAYTNAYKVELFLNGESLGERSYENKKTSWGAPYKETKDGKTYLEWAVPFKAGTLEAVAKDESGKEIARDQVVTAGSPAAVKLTADRKVISADGTDLSFITAEIVDSKGIVVPNADHLIKFNVSGQGELAGVDNGNASSVERYKDNKRKAFSGKAVAIIQSNKLAGEITVNASVAGLSGDTASLYTVAPADRDTKTVVGIDAVHVTVDVNEAPKLLSEIKVYYSDATVASKRVTWDAIDPKRYSTVGTFTIEGSVEGTSLKAKAFVTVKGIVAVKPYSTATKVGVQPVLVEKVTLLYSDETTKDVNVTWEDIAADQLAKEGRFVVEGSVEGTDLKAKAFVRVTNESKQVNIMLPAQGSTYPKLEATFTNPDDNLQHLNDGIKSYNNNPVNRWTNWTRTPRDAGDSITVNFDKQHVINNLDLFVFTDSGTVVPNKAAVQYWDGTAWKDVENLTQPSPYSVEKNEIRFDAVSTDKLKFHLTPSVKGKFLALTEAEIFADQI

SEQ ID NO: 11 - protein, 1313 aa, Neobacillus mesonae
MSKTTSAAGNSVNYDGERRMNFNENWRFQRETNGSIAGAQNPGFDDSSWRQLNLPHDWSIELDFNKNSLATHEGGYLDGGIGWYRKTFTIPESMKGKRISLDFDGVYMNSTTYLNGEMLGTYPFGYNAFSYDITDKLYKDGRPNVLVVKVNNTQPSSRWYSGSGIYRNVYLTVTDPIHVARYGTFVTTPNLEKTIKEDRADVNIKTKISNDSVETKQVKIKSTIYDEAGNAVQTVESEEKAAAAGTVTPFEQNTVIKQPKLWSISKPYRYRLVTEVIVGGQTVDTYETKFGARYFKFDENEGFSLNGEYMKLHGVSMHHDLGALGAATNARGVERQMQIMKDMGVNAIRVTHNPASPELLEAANKLGLFIVEEAFDSWAQSKKTYDYGRFFNSWAEHDIKEMVDRGKNEPAIIMWSIGNEIYDTTNATGVETARNLVRWVKEIDTTRPTTIGEDKTRGDKVNVTPINRYIKEIFDIVDVVGLNYSENNYDGYHKQNPNWKLYGSETSSATRSRGVYTHPYQNNQSTKYPDLQQSSYDNDYVGWGRTAEDAWKYDRDLKHIAGQFIWTGFDYIGEPTPYYNSYPAKSSYFGAVDTAGFPKDIFYYYQSQWKKEPMVHLLPHWNWKEGEKVRVLAYTNASKVELFLNGESLGEKGYENKQTSWGASYKETKDGKTYLEWAVPFKPGKLEAVAKDENGKVIARDQVVTAGEPAAVRLMADRKVVKADGTDLSFITAEIVDSKGIVVPNADHLIKFNVTGQGELAGVDNGNASSVERYKDNKRKAFSGKALAIVQSSKLSGKMTVHASVAGLSSDSTSVFTVTPADHDQKTAAGMDDVRLTVDVNEAPKLPSEIKVYYSDESAAVKKVTWDAVDPKQYSTVGEFTVEGSVEGTSLKAKAFVIVKGIVAVKPYSTATKVGVQPVLPEKATLLYSDETTKAAAVTWDEIASDKLAKEGQIVVEGSVEGTDLKAKAYVRVTNEVKSVNIMLQEQGSAYPKLEATFTNPDDNLQHLNDGIKSYNNNPVNRWTNWTRAPRDAGDSITVDFGKKHVIDNLDLFVFTDSGTVVPEKAAVQYWDGTAWKDVENLTQPSPYVVEKNKLRFDAVETDKMKFHLTPSVKGKFLALTEAEVYADQIAMGASAKLENITVNGKALEGFDPAKKNYELVLPYGSELPKIEAAAADNATVTILPAFSYPGTVKLFVTSEDGKITSEYSIRVSTEEPKLVSAELTVDKTNLIEDDVIDLKVIGLFESKEKIDVTDSQPTYEFDQQIVKIEGNKLYALEAGKVEVKATVTYKGVSVTTPAVTFTIAKNPAPKYI

SEQ ID NO: 12 - protein, 1309 aa, Neobacillus niacini
TSTTENSVKYEGERRINFNENWRFQRETNGSIAGAQNPGFDDSSWRRLNLPHDWSIELDFNKNSLATHEGGYLDGGIGWYRKTFTVPEAMKGKRISIDFDGVYMNSTTYLNGQLLGTYPFGYNAFSYDLTDKLYTDGRENVLVVKVNNTQPSSRWYSGSGIYRNVYLTVTNPVHVARYGTFVTTPDLETAYAEGEADVNIKTKVSNDSGEAAQVKVKSTIYDESGKAVSTVESEEKTAAAGTAANFDNNTIIEQPKLWSTDNPYRYKLVTEVIVGVQTVDTYETSFGARYFKFDENEGFSLNGTYMKLHGVSMHHDLGALGAATNARAVERQMQIMKDMGVNAIRVTHNPASPELLEAANKLGLFIVEEAFDSWAQSKKTYDYGRFFTTWAEHDIKEMVDRGKNEPAIIMWSIGNEIYDTTNAAGVETARNLVRWVKEIDTTRPTTIGEDKTRGDKVNVTPINSYIKEIFNIVDIVGLNYSENNYAGYHQQNPNWKLYGSETSSATRSRGVYTHPYQYNQSTKYPDLQQSSYDNDYVGWGRTAEDAWKYDRDLKHIAGQFIWTGFDYIGEPTPYYNSYPAKSSYFGAVDTAGFPKDIFYYYQSQWKKEPMVHLLPHWNWTEGEKVRVLAYTNAYKVELFLNGESLGERSYENKKTSWGAPYKETKDGKTYLEWAVPFKAGKLEAVAKDENGNEIGRDQEVTAGEPAAVKLTADRKVISADGTDLSFITAEIVDNKGVVVPNADHLIKFNVSGQGELAGVDNGNASSVERYKDTKRKAFSGKALAIIQSNKLSGEITVNATAAGLSSDSTSLFTVSPADRDKKTAVGMDAVHMTVAVNEAPKLPSAIQVYYSDTSVDSKNVTWDEIDPKRYSSVGTFTVEGSVEGTSLKAKAFITVKGIVAVKPVSTATKIGVPPVLPEKVTLLYSDETTKEVNVTWEEILEDKLAKVGRFTVEGTVAETDSKAKVYVRVTNETKAVNIMLPAQGSSYPQLEATFTNPADNLQHLNDGIKSYTNSPVNRWTNWTRTPRDAGDSIIVNFGKTHVINNLDLFVFTDSGTVVPDKAAVQYWDGTAWKDVENLTQPSPYVVEKNEIRFDSVQTDKLKFHLAPSVKGKFLALTEAEVYADQIVMSSTAELSSMTVNGKALADFDAAKKNYELVLPYGSELPKIEAEAKDNATVTILPAFAYPGSAKLFVTSEDGQVTSEYSIQVSMEEPKLVSAELSANRTNLLEDDMIDLKVKGLFESKEIVDLTDSQTTYEFDKPIVKIEGNKLYALEAGEVKVKAAVTYKGVSVATPAVTFKIAKNPAPKTI

SEQ ID NO: 13 - protein, 1678 aa, Streptomyces cirratus
DETPVAVATEKVEKETPKEEAVDSKASEQPVTTETVNSEAVETNHEVEKKVEAPTTETTPEKKETSDVEKQAPAVTQDQSAQTEKPELKPATNDEVKQLIEDRKEEFNQNWHFKLNANAKDAVKPDADVSSWKKLDLPHDWSIYNDFDHDSPAQNEGGQLNGGDAWYRKTFKLDEEDLNKNVRITFDGVYMDSQVYVNGQLVGHYPNGYNQFSYDITDYLHKDGRENVVAVHAINKQPSSRWYSGSGIYRDVTLQVTDKVHTEKNGTTILTPDLEKQQNGKVDTHVTSKIVNTDDKDHEILAEYQIIERNGQAVTDLVRTASQVLKAHQSASLNAILQVDKPKLWTVNSDKPALYELVTRVYRDGQLVDAKKDLFGYRYYNWTPNEGFSLNGERIKFHGVSLHHDHGALGAEENYKAEYRRLKQMKDMGVNSIRTTHNPASEQTLQIAAELGLLVQEEAFDTWYGGKKQYDYGRFFDKDATHPDAKKGEKWSDFDLRTMVERGKNNPAIVMWSIGNEIGEADGKPRSLATVKRLVQVIKAVDKTRYVTMGADKFRFGDGSGDHEKIANELDAVGFNYSEDNYKKLRAKHPNWLIYGSETSSATRTRGSYFRPERELVHSNQAYRHYEQSDYGNDRVGWGKTATASWTFDRDNAGYAGQFIWTGTDYIGEPTPWHNQNQTPVKSSYFGIVDTAGIPKNDYYLYQSQWVSAQKKPMVHLLPHWNWENPTLKANVADADGNIPVRAYSNAVSVELFLNGNTLGKKTFTKKQTSDGRTYQEGANANELYLEWKVAFEPGTLEAVARDEAGNIVARDKIVTAGEPAGVRLVKEDHAIAADGKDLTYIYYEIVDSKGNVVPTANNLVRFQLHGQGQIVGVDNGEQASRERYKEQADGSWIRKAFNGKGVVIVKSTEQAGKFTLTAHSDFLKSGQTTIFTGKKDQEEKTVLGTEVPKVRTVIGQAAKMPLKVGFIYSDGSRAKLPVEWSAVDVNQPGIFTVKGVAEGRDVEARVEVLALEAELPVVKRIAPSTDLSTVDPSVSYVLSDGTLGSYDVDRWEVAAEDQAKLTIPGSRIQAKGISGDDEIAATFVVAEGQAASPVVPTVTVADQPVEGLSTDQPVLYHKLAYGTALPEVKALAENAQVTVIQANEANGMRASIYVQPNDGGALQTYAIQFLQEAPQIERLSLEVENADALKEDQTVGIKVLAHYQDGTQAVLKADKVTFSTSGEGDVAVRKGMLELHKPGQVTLKAQFEGAEGQIDLNIQANTENKVVQAIRPVSVVTGLNQEPSLPDTVTVEYDKGFPKVHKVTWQAVAKEDLAKYHSFDVLGKVEGIENEAHAKVSVEGIIAVEEVTTTTPVSEAPQLPESVRTYHSNGQVSSAKVTWDAIDPSQYAQEGSFTVTGHVEGTQLPTKLHVRVSTQTETGANISDQWTGSELPLAFASDSNPSDSVANVNDKLISFNDQPANRWTNWNRTSEASVGILFGDSGILSKRSVDNLNVAFHEDHGVGAPKSYVIEYYVGKDVPTVPKNPSFVASEDHVFNDDNNWKQVTNLKAPNQVRAGEMTHFSFDKVNTYAVRIRMVRPDGKWGTSITEIQIFSKQVAAAKKAQAQIQVDGKDLPNFNPGLTDYYLEAKEGQAPTVTASVSDNGIATVIPSVREGDPVRVVVKAENGDILGEYRLHFT

SEQ ID NO: 14 - protein, 27 aa, Bacillus clausii
  SIGNAL 1..27
MKKPLGKIVASTALLISVAFSSSIASA

SEQ ID NO: 15 - protein, 8 aa, synthetic construct
HHHHHHPR